European Patent Application EP 4 717 702 A2, published April 1, 2026. Title: CELL-PENETRATING PEPTIDE CONJUGATES AND METHODS OF THEIR USE. Applicant: Oxford University Innovation Limited. The sequence listing filed with the application follows.

SEQUENCE LISTING (230 sequences)

SEQ ID NO: 1 - protein, 7 aa, synthetic construct
  MOD_RES 2: note = misc_feature - Xaa is bAla
  MOD_RES 5: note = misc_feature - Xaa is bAla
RXRRXRR

SEQ ID NO: 2-3 - skipped (2 entries)

SEQ ID NO: 4 - protein, 6 aa, synthetic construct
  MOD_RES 2: note = misc_feature - Xaa is bAla
  MOD_RES 5: note = misc_feature - Xaa is bAla
RXRRXR

SEQ ID NO: 5 - protein, 6 aa, synthetic construct
  MOD_RES 3: note = misc_feature - Xaa is bAla
  MOD_RES 5: note = misc_feature - Xaa is bAla
RRXRXR

SEQ ID NO: 6-9 - skipped (4 entries)

SEQ ID NO: 10 - protein, 7 aa, synthetic construct
  MOD_RES 2: note = misc_feature - Xaa is bAla
  MOD_RES 5: note = misc_feature - Xaa is bAla
RXRHXHR

SEQ ID NO: 11 - protein, 7 aa, synthetic construct
  MOD_RES 2: note = misc_feature - Xaa is bAla
  MOD_RES 4..5: note = misc_feature - Xaa is bAla
RXRXXHR

SEQ ID NO: 12 - protein, 6 aa, synthetic construct
  MOD_RES 2: note = misc_feature - Xaa is bAla
  MOD_RES 5: note = misc_feature - Xaa is bAla
RXRRXH

SEQ ID NO: 13 - protein, 6 aa, synthetic construct
  MOD_RES 2: note = misc_feature - Xaa is bAla
  MOD_RES 5: note = misc_feature - Xaa is bAla
HXRRXR

SEQ ID NO: 14-18 - skipped (5 entries)

SEQ ID NO: 19 - protein, 6 aa, synthetic construct
  MOD_RES 2: note = misc_feature - Xaa is hydroxyproline
  MOD_RES 5: note = misc_feature - Xaa is hydroxyproline
RXRRXR

SEQ ID NO: 20 - protein, 5 aa, synthetic construct
YQFLI

SEQ ID NO: 21 - protein, 5 aa, synthetic construct
FQILY

SEQ ID NO: 22 - protein, 5 aa, synthetic construct
ILFQY

SEQ ID NO: 23 - protein, 4 aa, synthetic construct
FQIY

SEQ ID NO: 24 - protein, 5 aa, synthetic construct
WWPWW

SEQ ID NO: 25 - protein, 4 aa, synthetic construct
WPWW

SEQ ID NO: 26 - protein, 4 aa, synthetic construct
WWPW

SEQ ID NO: 27 - protein, 17 aa, synthetic construct
  MOD_RES 2: note = misc_feature - Xaa is bAla
  MOD_RES 5: note = misc_feature - Xaa is bAla
  MOD_RES 14: note = misc_feature - Xaa is bAla
  MOD_RES 16: note = misc_feature - Xaa is bAla
RXRRXRRFQILYRXRXR

SEQ ID NO: 28 - protein, 16 aa, synthetic construct
  MOD_RES 2: note = misc_feature - Xaa is bAla
  MOD_RES 5: note = misc_feature - Xaa is bAla
  MOD_RES 14: note = misc_feature - Xaa is bAla
RXRRXRRFQILYRXRR

SEQ ID NO: 29 - protein, 17 aa, synthetic construct
  MOD_RES 2: note = misc_feature - Xaa is bAla
  MOD_RES 5: note = misc_feature - Xaa is bAla
  MOD_RES 14: note = misc_feature - Xaa is bAla
  MOD_RES 16: note = misc_feature - Xaa is bAla
RXRRXRFQILYRRXRXR

SEQ ID NO: 30 - protein, 17 aa, synthetic construct
  MOD_RES 2: note = misc_feature - Xaa is bAla
  MOD_RES 4: note = misc_feature - Xaa is bAla
  MOD_RES 12: note = misc_feature - Xaa is bAla
  MOD_RES 15: note = misc_feature - Xaa is bAla
RXRXRFQILYRXRRXRR

SEQ ID NO: 31 - protein, 17 aa, synthetic construct
  MOD_RES 2: note = misc_feature - Xaa is bAla
  MOD_RES 5: note = misc_feature - Xaa is bAla
  MOD_RES 14: note = misc_feature - Xaa is bAla
  MOD_RES 16: note = misc_feature - Xaa is bAla
RXRRXRRYQFLIRXRXR

SEQ ID NO: 32 - protein, 17 aa, synthetic construct
  MOD_RES 2: note = misc_feature - Xaa is bAla
  MOD_RES 5: note = misc_feature - Xaa is bAla
  MOD_RES 14: note = misc_feature - Xaa is bAla
  MOD_RES 16: note = misc_feature - Xaa is bAla
RXRRXRRILFQYRXRXR

SEQ ID NO: 33 - protein, 16 aa, synthetic construct
  MOD_RES 2: note = misc_feature - Xaa is bAla
  MOD_RES 5: note = misc_feature - Xaa is bAla
  MOD_RES 13: note = misc_feature - Xaa is bAla
  MOD_RES 15: note = misc_feature - Xaa is bAla
RXRRXRFQILYRXRXR

SEQ ID NO: 34 - protein, 16 aa, synthetic construct
  MOD_RES 2: note = misc_feature - Xaa is bAla
  MOD_RES 5: note = misc_feature - Xaa is bAla
  MOD_RES 12: note = misc_feature - Xaa is bAla
  MOD_RES 15: note = misc_feature - Xaa is bAla
RXRRXFQILYRXRRXR

SEQ ID NO: 35 - protein, 15 aa, synthetic construct
  MOD_RES 2: note = misc_feature - Xaa is bAla
  MOD_RES 5: note = misc_feature - Xaa is bAla
  MOD_RES 12: note = misc_feature - Xaa is bAla
  MOD_RES 14: note = misc_feature - Xaa is bAla
RXRRXRFQILYXRXR

SEQ ID NO: 36 - protein, 15 aa, synthetic construct
  MOD_RES 2: note = misc_feature - Xaa is bAla
  MOD_RES 5: note = misc_feature - Xaa is bAla
  MOD_RES 12: note = misc_feature - Xaa is bAla
  MOD_RES 14: note = misc_feature - Xaa is bAla
RXRRXFQILYRXRXR

SEQ ID NO: 37 - protein, 17 aa, synthetic construct
  MOD_RES 2: note = misc_feature - Xaa is bAla
  MOD_RES 5: note = misc_feature - Xaa is bAla
  MOD_RES 14: note = misc_feature - Xaa is bAla
  MOD_RES 16: note = misc_feature - Xaa is bAla
RXRRXRRFQILYRXHXH

SEQ ID NO: 38 - protein, 17 aa, synthetic construct
  MOD_RES 2: note = misc_feature - Xaa is bAla
  MOD_RES 5: note = misc_feature - Xaa is bAla
  MOD_RES 14: note = misc_feature - Xaa is bAla
  MOD_RES 16: note = misc_feature - Xaa is bAla
RXRRXRRFQILYHXHXR

SEQ ID NO: 39 - protein, 17 aa, synthetic construct
  MOD_RES 2: note = misc_feature - Xaa is bAla
  MOD_RES 5: note = misc_feature - Xaa is bAla
  MOD_RES 14: note = misc_feature - Xaa is bAla
  MOD_RES 16: note = misc_feature - Xaa is bAla
RXRRXRRFQILYHXRXH

SEQ ID NO: 40 - protein, 17 aa, synthetic construct
  MOD_RES 2: note = misc_feature - Xaa is bAla
  MOD_RES 5: note = misc_feature - Xaa is bAla
  MOD_RES 14: note = misc_feature - Xaa is bAla
  MOD_RES 16: note = misc_feature - Xaa is bAla
RXRRXRRYQFLIRXHXH

SEQ ID NO: 41 - protein, 17 aa, synthetic construct
  MOD_RES 2: note = misc_feature - Xaa is bAla
  MOD_RES 5: note = misc_feature - Xaa is bAla
  MOD_RES 14: note = misc_feature - Xaa is bAla
  MOD_RES 16: note = misc_feature - Xaa is bAla
RXRRXRRILFQYRXHXH

SEQ ID NO: 42 - protein, 17 aa, synthetic construct
  MOD_RES 2: note = misc_feature - Xaa is bAla
  MOD_RES 5: note = misc_feature - Xaa is bAla
  MOD_RES 14: note = misc_feature - Xaa is bAla
  MOD_RES 16: note = misc_feature - Xaa is bAla
RXRHXHRFQILYRXRXR

SEQ ID NO: 43 - protein, 17 aa, synthetic construct
  MOD_RES 2: note = misc_feature - Xaa is bAla
  MOD_RES 4: note = misc_feature - Xaa is bAla
  MOD_RES 5: note = misc_feature - Xaa is bAla
  MOD_RES 14: note = misc_feature - Xaa is bAla
  MOD_RES 16: note = misc_feature - Xaa is bAla
RXRXXHRFQILYRXHXH

SEQ ID NO: 44 - protein, 16 aa, synthetic construct
  MOD_RES 2: note = misc_feature - Xaa is bAla
  MOD_RES 5: note = misc_feature - Xaa is bAla
  MOD_RES 13: note = misc_feature - Xaa is bAla
  MOD_RES 15: note = misc_feature - Xaa is bAla
RXRRXRFQILYRXHXH

SEQ ID NO: 45 - protein, 16 aa, synthetic construct
  MOD_RES 2: note = misc_feature - Xaa is bAla
  MOD_RES 5: note = misc_feature - Xaa is bAla
  MOD_RES 13: note = misc_feature - Xaa is bAla
  MOD_RES 15: note = misc_feature - Xaa is bAla
RXRRXRFQILYHXHXH

SEQ ID NO: 46 - protein, 16 aa, synthetic construct
  MOD_RES 2: note = misc_feature - Xaa is bAla
  MOD_RES 5: note = misc_feature - Xaa is bAla
  MOD_RES 13: note = misc_feature - Xaa is bAla
  MOD_RES 15: note = misc_feature - Xaa is bAla
RXRRXHFQILYRXHXH

SEQ ID NO: 47 - protein, 16 aa, synthetic construct
  MOD_RES 2: note = misc_feature - Xaa is bAla
  MOD_RES 5: note = misc_feature - Xaa is bAla
  MOD_RES 13: note = misc_feature - Xaa is bAla
  MOD_RES 15: note = misc_feature - Xaa is bAla
HXRRXRFQILYRXHXH

SEQ ID NO: 48 - protein, 15 aa, synthetic construct
  MOD_RES 2: note = misc_feature - Xaa is bAla
  MOD_RES 5: note = misc_feature - Xaa is bAla
  MOD_RES 12: note = misc_feature - Xaa is bAla
  MOD_RES 14: note = misc_feature - Xaa is bAla
RXRRXFQILYRXHXH

SEQ ID NO: 49 - protein, 15 aa, synthetic construct
  MOD_RES 2: note = misc_feature - Xaa is bAla
  MOD_RES 5: note = misc_feature - Xaa is bAla
  MOD_RES 12: note = misc_feature - Xaa is bAla
  MOD_RES 14: note = misc_feature - Xaa is bAla
RXRRXRFQILYXHXH

SEQ ID NO: 50 - protein, 16 aa, synthetic construct
  MOD_RES 2: note = misc_feature - Xaa is bAla
  MOD_RES 5: note = misc_feature - Xaa is bAla
  MOD_RES 13: note = misc_feature - Xaa is bAla
  MOD_RES 15: note = misc_feature - Xaa is bAla
RXRRXRYQFLIHXHXH

SEQ ID NO: 51 - protein, 16 aa, synthetic construct
  MOD_RES 2: note = misc_feature - Xaa is bAla
  MOD_RES 5: note = misc_feature - Xaa is bAla
  MOD_RES 13: note = misc_feature - Xaa is bAla
  MOD_RES 15: note = misc_feature - Xaa is bAla
RXRRXRILFQYHXHXH

SEQ ID NO: 52 - protein, 17 aa, synthetic construct
  MOD_RES 2: note = misc_feature - Xaa is bAla
  MOD_RES 5: note = misc_feature - Xaa is bAla
  MOD_RES 14: note = misc_feature - Xaa is bAla
  MOD_RES 16: note = misc_feature - Xaa is bAla
RXRRXRRFQILYHXHXH

SEQ ID NO: 53 - protein, 15 aa, synthetic construct
  MOD_RES 2: note = misc_feature - Xaa is bAla
  MOD_RES 5: note = misc_feature - Xaa is bAla
  MOD_RES 12: note = misc_feature - Xaa is bAla
  MOD_RES 14: note = misc_feature - Xaa is bAla
RXRRXRFQILYXRXS

SEQ ID NO: 54 - protein, 15 aa, synthetic construct
  MOD_RES 2: note = misc_feature - Xaa is bAla
  MOD_RES 5: note = misc_feature - Xaa is bAla
  MOD_RES 12: note = misc_feature - Xaa is bAla
  MOD_RES 14: note = misc_feature - Xaa is bAla
  MOD_RES 15: note = misc_feature - Xaa is hydroxyproline
RXRRXRFQILYXRXX

SEQ ID NO: 55 - protein, 15 aa, synthetic construct
  MOD_RES 2: note = misc_feature - Xaa is bAla
  MOD_RES 5: note = misc_feature - Xaa is bAla
  MOD_RES 12: note = misc_feature - Xaa is bAla
  MOD_RES 14: note = misc_feature - Xaa is hydroxyproline
RXRRXRFQILYXRXR

SEQ ID NO: 56 - protein, 16 aa, synthetic construct
  MOD_RES 3: note = misc_feature - Xaa is bAla
  MOD_RES 6: note = misc_feature - Xaa is bAla
  MOD_RES 13: note = misc_feature - Xaa is bAla
  MOD_RES 15: note = misc_feature - Xaa is bAla
RRXRRXRFQILYXRXR

SEQ ID NO: 57 - protein, 15 aa, synthetic construct
  MOD_RES 1: note = misc_feature - Xaa is bAla
  MOD_RES 4: note = misc_feature - Xaa is bAla
  MOD_RES 12: note = misc_feature - Xaa is bAla
  MOD_RES 14: note = misc_feature - Xaa is bAla
XRRXRRFQILYXRXR

SEQ ID NO: 58 - protein, 13 aa, synthetic construct
  MOD_RES 2: note = misc_feature - Xaa is bAla
  MOD_RES 5: note = misc_feature - Xaa is bAla
  MOD_RES 10: note = misc_feature - Xaa is bAla
  MOD_RES 12: note = misc_feature - Xaa is bAla
RXRRXRWWWXRXR

SEQ ID NO: 59 - protein, 15 aa, synthetic construct
  MOD_RES 2: note = misc_feature - Xaa is bAla
  MOD_RES 5: note = misc_feature - Xaa is bAla
  MOD_RES 12: note = misc_feature - Xaa is bAla
  MOD_RES 14: note = misc_feature - Xaa is bAla
RXRRXRWWPWWXRXR

SEQ ID NO: 60 - protein, 14 aa, synthetic construct
  MOD_RES 2: note = misc_feature - Xaa is bAla
  MOD_RES 5: note = misc_feature - Xaa is bAla
  MOD_RES 11: note = misc_feature - Xaa is bAla
  MOD_RES 13: note = misc_feature - Xaa is bAla
RXRRXRWPWWXRXR

SEQ ID NO: 61 - protein, 14 aa, synthetic construct
  MOD_RES 2: note = misc_feature - Xaa is bAla
  MOD_RES 5: note = misc_feature - Xaa is bAla
  MOD_RES 11: note = misc_feature - Xaa is bAla
  MOD_RES 13: note = misc_feature - Xaa is bAla
RXRRXRWWPWXRXR

SEQ ID NO: 62 - protein, 15 aa, synthetic construct
  MOD_RES 2: note = misc_feature - Xaa is bAla
  MOD_RES 5: note = misc_feature - Xaa is bAla
  MOD_RES 12: note = misc_feature - Xaa is bAla
  MOD_RES 14: note = misc_feature - Xaa is bAla
RXRRXRRWWWRXRXR

SEQ ID NO: 63 - protein, 17 aa, synthetic construct
  MOD_RES 2: note = misc_feature - Xaa is bAla
  MOD_RES 5: note = misc_feature - Xaa is bAla
  MOD_RES 14: note = misc_feature - Xaa is bAla
  MOD_RES 16: note = misc_feature - Xaa is bAla
RXRRXRRWWPWWRXRXR

SEQ ID NO: 64 - protein, 16 aa, synthetic construct
  MOD_RES 2: note = misc_feature - Xaa is bAla
  MOD_RES 5: note = misc_feature - Xaa is bAla
  MOD_RES 13: note = misc_feature - Xaa is bAla
  MOD_RES 15: note = misc_feature - Xaa is bAla
RXRRXRRWPWWRXRXR

SEQ ID NO: 65 - protein, 16 aa, synthetic construct
  MOD_RES 2: note = misc_feature - Xaa is bAla
  MOD_RES 5: note = misc_feature - Xaa is bAla
  MOD_RES 13: note = misc_feature - Xaa is bAla
  MOD_RES 15: note = misc_feature - Xaa is bAla
RXRRXRRWWPWRXRXR

SEQ ID NO: 66 - protein, 16 aa, synthetic construct
  MOD_RES 2: note = misc_feature - Xaa is bAla
  MOD_RES 5: note = misc_feature - Xaa is bAla
  MOD_RES 13: note = misc_feature - Xaa is bAla
  MOD_RES 15: note = misc_feature - Xaa is bAla
RXRRXRRFQILYXRXR

SEQ ID NO: 67 - protein, 15 aa, synthetic construct
  MOD_RES 2: note = misc_feature - Xaa is bAla
  MOD_RES 5: note = misc_feature - Xaa is bAla
  MOD_RES 14: note = misc_feature - Xaa is bAla
RXRRXRRFQILYRXR

SEQ ID NO: 68 - protein, 16 aa, synthetic construct
  MOD_RES 1: note = misc_feature - Xaa is bAla
  MOD_RES 3: note = misc_feature - Xaa is bAla
  MOD_RES 5: note = misc_feature - Xaa is bAla
  MOD_RES 12: note = misc_feature - Xaa is bAla
  MOD_RES 15: note = misc_feature - Xaa is bAla
XRXRXWWPWWRXRRXR

SEQ ID NO: 69 - protein, 16 aa, synthetic construct
  MOD_RES 2: note = misc_feature - Xaa is bAla
  MOD_RES 5: note = misc_feature - Xaa is bAla
  MOD_RES 13: note = misc_feature - Xaa is bAla
  MOD_RES 15: note = misc_feature - Xaa is bAla
RXRRXRRFQILYXHXH

SEQ ID NO: 70 - protein, 16 aa, synthetic construct
  MOD_RES 2: note = misc_feature - Xaa is bAla
  MOD_RES 5: note = misc_feature - Xaa is bAla
  MOD_RES 13: note = misc_feature - Xaa is bAla
  MOD_RES 15: note = misc_feature - Xaa is bAla
RXRRXRRFQIYRXHXH

SEQ ID NO: 71 - protein, 15 aa, synthetic construct
  MOD_RES 2: note = misc_feature - Xaa is bAla
  MOD_RES 5: note = misc_feature - Xaa is bAla
  MOD_RES 12: note = misc_feature - Xaa is bAla
  MOD_RES 14: note = misc_feature - Xaa is bAla
RXRRXRFQILYXRXH

SEQ ID NO: 72 - protein, 16 aa, synthetic construct
  MOD_RES 2: note = misc_feature - Xaa is bAla
  MOD_RES 5: note = misc_feature - Xaa is bAla
  MOD_RES 13: note = misc_feature - Xaa is hydroxyproline
  MOD_RES 15: note = misc_feature - Xaa is hydroxyproline
RXRRXRFQILYRXHXH

SEQ ID NO: 73 - protein, 16 aa, synthetic construct
  MOD_RES 2: note = misc_feature - Xaa is hydroxyproline
  MOD_RES 5: note = misc_feature - Xaa is hydroxyproline
  MOD_RES 13: note = misc_feature - Xaa is bAla
  MOD_RES 15: note = misc_feature - Xaa is bAla
RXRRXRFQILYRXHXH

SEQ ID NO: 74 - protein, 16 aa, synthetic construct
  MOD_RES 2: note = misc_feature - Xaa is hydroxyproline
  MOD_RES 5: note = misc_feature - Xaa is hydroxyproline
  MOD_RES 13: note = misc_feature - Xaa is hydroxyproline
  MOD_RES 15: note = misc_feature - Xaa is hydroxyproline
RXRRXRFQILYRXHXH

SEQ ID NO: 75 - protein, 14 aa, synthetic construct
  MOD_RES 2: note = misc_feature - Xaa is bAla
  MOD_RES 5: note = misc_feature - Xaa is bAla
  MOD_RES 11: note = misc_feature - Xaa is bAla
  MOD_RES 13: note = misc_feature - Xaa is bAla
RXRRXRWWWRXHXH

SEQ ID NO: 76 - protein, 14 aa, synthetic construct
  MOD_RES 2: note = misc_feature - Xaa is bAla
  MOD_RES 5: note = misc_feature - Xaa is bAla
  MOD_RES 11: note = misc_feature - Xaa is bAla
  MOD_RES 13: note = misc_feature - Xaa is bAla
RXRRXRWWPRXHXH

SEQ ID NO: 77 - protein, 14 aa, synthetic construct
  MOD_RES 2: note = misc_feature - Xaa is bAla
  MOD_RES 5: note = misc_feature - Xaa is bAla
  MOD_RES 11: note = misc_feature - Xaa is bAla
  MOD_RES 13: note = misc_feature - Xaa is bAla
RXRRXRPWWRXHXH

SEQ ID NO: 78 - protein, 16 aa, synthetic construct
  MOD_RES 2: note = misc_feature - Xaa is bAla
  MOD_RES 5: note = misc_feature - Xaa is bAla
  MOD_RES 13: note = misc_feature - Xaa is bAla
  MOD_RES 15: note = misc_feature - Xaa is bAla
RXRRXRWWPWWRXHXH

SEQ ID NO: 79 - protein, 15 aa, synthetic construct
  MOD_RES 2: note = misc_feature - Xaa is bAla
  MOD_RES 5: note = misc_feature - Xaa is bAla
  MOD_RES 12: note = misc_feature - Xaa is bAla
  MOD_RES 14: note = misc_feature - Xaa is bAla
RXRRXRWWPWRXHXH

SEQ ID NO: 80 - protein, 15 aa, synthetic construct
  MOD_RES 2: note = misc_feature - Xaa is bAla
  MOD_RES 5: note = misc_feature - Xaa is bAla
  MOD_RES 12: note = misc_feature - Xaa is bAla
  MOD_RES 14: note = misc_feature - Xaa is bAla
RXRRXRWPWWRXHXH

SEQ ID NO: 81 - protein, 15 aa, synthetic construct
  MOD_RES 2: note = misc_feature - Xaa is bAla
  MOD_RES 5: note = misc_feature - Xaa is bAla
  MOD_RES 12: note = misc_feature - Xaa is bAla
  MOD_RES 14: note = misc_feature - Xaa is bAla
RXRRXRRWWWRXHXH

SEQ ID NO: 82 - protein, 17 aa, synthetic construct
  MOD_RES 2: note = misc_feature - Xaa is bAla
  MOD_RES 5: note = misc_feature - Xaa is bAla
  MOD_RES 14: note = misc_feature - Xaa is bAla
  MOD_RES 16: note = misc_feature - Xaa is bAla
RXRRXRRWWPWWRXHXH

SEQ ID NO: 83 - protein, 16 aa, synthetic construct
  MOD_RES 2: note = misc_feature - Xaa is bAla
  MOD_RES 5: note = misc_feature - Xaa is bAla
  MOD_RES 13: note = misc_feature - Xaa is bAla
  MOD_RES 15: note = misc_feature - Xaa is bAla
RXRRXRRWPWWRXHXH

SEQ ID NO: 84 - protein, 16 aa, synthetic construct
  MOD_RES 2: note = misc_feature - Xaa is bAla
  MOD_RES 5: note = misc_feature - Xaa is bAla
  MOD_RES 13: note = misc_feature - Xaa is bAla
  MOD_RES 15: note = misc_feature - Xaa is bAla
RXRRXRRWWPWRXHXH

SEQ ID NO: 85 - protein, 17 aa, synthetic construct
  MOD_RES 3: note = misc_feature - Xaa is bAla
  MOD_RES 6: note = misc_feature - Xaa is bAla
  MOD_RES 14: note = misc_feature - Xaa is bAla
  MOD_RES 16: note = misc_feature - Xaa is bAla
RRXRRXRFQILYRXHXH

SEQ ID NO: 86 - protein, 16 aa, synthetic construct
  MOD_RES 1: note = misc_feature - Xaa is bAla
  MOD_RES 4: note = misc_feature - Xaa is bAla
  MOD_RES 13: note = misc_feature - Xaa is bAla
  MOD_RES 15: note = misc_feature - Xaa is bAla
XRRXRRFQILYRXHXH

SEQ ID NO: 87 - protein, 16 aa, synthetic construct
  MOD_RES 3: note = misc_feature - Xaa is bAla
  MOD_RES 6: note = misc_feature - Xaa is bAla
  MOD_RES 13: note = misc_feature - Xaa is bAla
  MOD_RES 15: note = misc_feature - Xaa is bAla
RRXRRXRFQILYXHXH

SEQ ID NO: 88 - protein, 15 aa, synthetic construct
  MOD_RES 1: note = misc_feature - Xaa is bAla
  MOD_RES 4: note = misc_feature - Xaa is bAla
  MOD_RES 12: note = misc_feature - Xaa is bAla
  MOD_RES 14: note = misc_feature - Xaa is bAla
XRRXRRFQILYXHXH

SEQ ID NO: 89 - protein, 17 aa, synthetic construct
  MOD_RES 2: note = misc_feature - Xaa is bAla
  MOD_RES 5: note = misc_feature - Xaa is bAla
  MOD_RES 14: note = misc_feature - Xaa is bAla
  MOD_RES 16: note = misc_feature - Xaa is bAla
RXRRXHRFQILYRXHXH

SEQ ID NO: 90 - DNA, 25 bp, synthetic construct
  source 1..25: mol_type = other DNA
ggccaaacctcggcttacctgaaat

SEQ ID NO: 91 - DNA, 22 bp, synthetic construct
  source 1..22: mol_type = other DNA
cagaattctgccaattgctgag

SEQ ID NO: 92 - DNA, 20 bp, synthetic construct
  source 1..20: mol_type = other DNA
ttcttcagcttgtgtcatcc

SEQ ID NO: 93 - DNA, 24 bp, synthetic construct
  source 1..24: mol_type = other DNA
cccagtctaccaccctatcagagc

SEQ ID NO: 94 - DNA, 20 bp, synthetic construct
  source 1..20: mol_type = other DNA
cctgcctttaaggcttcctt

SEQ ID NO: 95 - DNA, 20 bp, synthetic construct
  source 1..20: mol_type = other DNA
caggccattcctctttcagg

SEQ ID NO: 96 - DNA, 21 bp, synthetic construct
  source 1..21: mol_type = other DNA
gaaactttcctcccagttggt

SEQ ID NO: 97 - DNA, 29 bp, synthetic construct
  modified_base 1: mod_base = OTHER; note = misc_feature - Labelled with FAM
  modified_base 9..10: mod_base = OTHER; note = misc_feature - Residues no. 9 and no. 10 are linked through an internal quencher ZEN
  modified_base 29: mod_base = OTHER; note = misc_feature - Labelled with IABkFQ
  source 1..29: mol_type = other DNA
tcaacttcagccatccatttctgtaaggt

SEQ ID NO: 98 - DNA, 30 bp, synthetic construct
  source 1..30: mol_type = other DNA
ctgaatatgaaataatggaggagagactcg

SEQ ID NO: 99 - DNA, 25 bp, synthetic construct
  source 1..25: mol_type = other DNA
cttcagccatccatttctgtaaggt

SEQ ID NO: 100 - DNA, 19 bp, synthetic construct
  modified_base 1: mod_base = OTHER; note = misc_feature - Labelled with FAM
  modified_base 9..10: mod_base = OTHER; note = misc_feature - residues no. 9 and no. 10 are linked through an internal quencher ZEN
  modified_base 19: mod_base = OTHER; note = misc_feature - Labelled with IABkFQ
  source 1..19: mol_type = other DNA
atgtgattctgtaatttcc

SEQ ID NO: 101 - protein, 15 aa, synthetic construct
  MOD_RES 2: note = misc_feature - Xaa is bAla
  MOD_RES 5: note = misc_feature - Xaa is bAla
  MOD_RES 12: note = misc_feature - Xaa is hydroxyproline
  MOD_RES 14: note = misc_feature - Xaa is hydroxyproline
RXRRXRFQILYXRXR

SEQ ID NO: 102 - protein, 15 aa, synthetic construct
  MOD_RES 2: note = misc_feature - Xaa is hydroxyproline
  MOD_RES 5: note = misc_feature - Xaa is hydroxyproline
  MOD_RES 12: note = misc_feature - Xaa is bAla
  MOD_RES 14: note = misc_feature - Xaa is bAla
RXRRXRFQILYXRXR

SEQ ID NO: 103 - protein, 15 aa, synthetic construct
  MOD_RES 2: note = misc_feature - Xaa is hydroxyproline
  MOD_RES 5: note = misc_feature - Xaa is hydroxyproline
  MOD_RES 12: note = misc_feature - Xaa is hydroxyproline
  MOD_RES 14: note = misc_feature - Xaa is hydroxyproline
RXRRXRFQILYXRXR

SEQ ID NO: 104 - protein, 13 aa, synthetic construct
  MOD_RES 2: note = misc_feature - Xaa is bAla
  MOD_RES 5: note = misc_feature - Xaa is bAla
  MOD_RES 10: note = misc_feature - Xaa is bAla
  MOD_RES 12: note = misc_feature - Xaa is bAla
RXRRXRWWWXRXR

SEQ ID NO: 105 - protein, 15 aa, synthetic construct
  MOD_RES 2: note = misc_feature - Xaa is bAla
  MOD_RES 5: note = misc_feature - Xaa is bAla
  MOD_RES 12: note = misc_feature - Xaa is bAla
  MOD_RES 14: note = misc_feature - Xaa is bAla
RXRRXRWWPWWXRXR

SEQ ID NO: 106 - RNA, 30 nt, synthetic construct
  source 1..30: mol_type = other RNA
ccaatgccatcctggagttcctgtaagata

SEQ ID NO: 107 - RNA, 30 nt, synthetic construct
  source 1..30: mol_type = other RNA
gctgcccaatgccatcctggagttcctgta

SEQ ID NO: 108 - RNA, 27 nt, synthetic construct
  source 1..27: mol_type = other RNA
caatgccatcctggagttcctgtaaga

SEQ ID NO: 109 - RNA, 30 nt, synthetic construct; identical to SEQ ID NO: 107
  source 1..30: mol_type = other RNA

SEQ ID NO: 110 - RNA, 39 nt, synthetic construct
  source 1..39: mol_type = other RNA
gctgcccaatgccatcctggagttcctgtaagataccaa

SEQ ID NO: 111 - RNA, 30 nt, synthetic construct
  source 1..30: mol_type = other RNA
gcccaatgccatcctggagttcctgtaaga

SEQ ID NO: 112 - RNA, 28 nt, synthetic construct
  source 1..28: mol_type = other RNA
tgccatcctggagttcctgtaagatacc

SEQ ID NO: 113 - RNA, 25 nt, synthetic construct
  source 1..25: mol_type = other RNA
gcccaatgccatcctggagttcctg

SEQ ID NO: 114 - RNA, 28 nt, synthetic construct
  source 1..28: mol_type = other RNA
gctgcccaatgccatcctggagttcctg

SEQ ID NO: 115 - RNA, 25 nt, synthetic construct
  source 1..25: mol_type = other RNA
tgccatcctggagttcctgtaagat

SEQ ID NO: 116 - RNA, 28 nt, synthetic construct
  source 1..28: mol_type = other RNA
caatgccatcctggagttcctgtaagat

SEQ ID NO: 117 - RNA, 31 nt, synthetic construct
  source 1..31: mol_type = other RNA
gcccaatgccatcctggagttcctgtaagat

SEQ ID NO: 118 - RNA, 30 nt, synthetic construct
  source 1..30: mol_type = other RNA
ttgccgctgcccaatgccatcctggagttc

SEQ ID NO: 119 - RNA, 30 nt, synthetic construct; identical to SEQ ID NO: 107
  source 1..30: mol_type = other RNA

SEQ ID NO: 120 - RNA, 28 nt, synthetic construct
  source 1..28: mol_type = other RNA
gcccaatgccatcctggagttcctgtaa

SEQ ID NO: 121 - RNA, 30 nt, synthetic construct
  source 1..30: mol_type = other RNA
gccgctgcccaatgccatcctggagttcct

SEQ ID NO: 122 - RNA, 22 nt, synthetic construct
  source 1..22: mol_type = other RNA
caatgccatcctggagttcctg

SEQ ID NO: 123 - RNA, 31 nt, synthetic construct
  source 1..31: mol_type = other RNA
gctgcccaatgccatcctggagttcctgtaa

SEQ ID NO: 124 - RNA, 31 nt, synthetic construct
  source 1..31: mol_type = other RNA
caatgccatcctggagttcctgtaagatacc

SEQ ID NO: 125 - RNA, 26 nt, synthetic construct
  source 1..26: mol_type = other RNA
accagagtaacagtctgagtaggagc

SEQ ID NO: 126 - RNA, 23 nt, synthetic construct
  source 1..23: mol_type = other RNA
ctcataccttctgcttgatgatc

SEQ ID NO: 127 - RNA, 24 nt, synthetic construct
  source 1..24: mol_type = other RNA
ttctgtccaagcccggttgaaatc

SEQ ID NO: 128 - RNA, 30 nt, synthetic construct
  source 1..30: mol_type = other RNA
acatcaaggaagatggcatttctagtttgg

SEQ ID NO: 129 - RNA, 25 nt, synthetic construct
  source 1..25: mol_type = other RNA
acatcaaggaagatggcatttctag

SEQ ID NO: 130 - RNA, 30 nt, synthetic construct
  source 1..30: mol_type = other RNA
ctccaacatcaaggaagatggcatttctag

SEQ ID NO: 131 - RNA, 27 nt, synthetic construct
  source 1..27: mol_type = other RNA
atcattttttctcataccttctgctag

SEQ ID NO: 132 - RNA, 38 nt, synthetic construct
  source 1..38: mol_type = other RNA
atcattttttctcataccttctgctaggagctaaaaag

SEQ ID NO: 133 - RNA, 21 nt, synthetic construct
  source 1..21: mol_type = other RNA
cacccaccatcaccctctgtg

SEQ ID NO: 134 - RNA, 22 nt, synthetic construct
  source 1..22: mol_type = other RNA
atcatctcgttgatatcctcaa

SEQ ID NO: 135 - DNA, 23 bp, synthetic construct
  source 1..23: mol_type = other DNA
ccggttctgaaggtgttcttgta

SEQ ID NO: 136 - DNA, 24 bp, synthetic construct
  source 1..24: mol_type = other DNA
tccggttctgaaggtgttcttgta

SEQ ID NO: 137 - DNA, 25 bp, synthetic construct
  source 1..25: mol_type = other DNA
ctccggttctgaaggtgttcttgta

SEQ ID NO: 138 - DNA, 26 bp, synthetic construct
  source 1..26: mol_type = other DNA
cctccggttctgaaggtgttcttgta

SEQ ID NO: 139 - DNA, 27 bp, synthetic construct
  source 1..27: mol_type = other DNA
gcctccggttctgaaggtgttcttgta

SEQ ID NO: 140 - DNA, 28 bp, synthetic construct
  source 1..28: mol_type = other DNA
tgcctccggttctgaaggtgttcttgta

SEQ ID NO: 141 - DNA, 22 bp, synthetic construct
  source 1..22: mol_type = other DNA
ccggttctgaaggtgttcttgt

SEQ ID NO: 142 - DNA, 23 bp, synthetic construct
  source 1..23: mol_type = other DNA
tccggttctgaaggtgttcttgt

SEQ ID NO: 143 - DNA, 24 bp, synthetic construct
  source 1..24: mol_type = other DNA
ctccggttctgaaggtgttcttgt

SEQ ID NO: 144 - DNA, 25 bp, synthetic construct
  source 1..25: mol_type = other DNA
cctccggttctgaaggtgttcttgt

SEQ ID NO: 145 - DNA, 26 bp, synthetic construct
  source 1..26: mol_type = other DNA
gcctccggttctgaaggtgttcttgt

SEQ ID NO: 146 - DNA, 27 bp, synthetic construct
  source 1..27: mol_type = other DNA
tgcctccggttctgaaggtgttcttgt

SEQ ID NO: 147 - DNA, 21 bp, synthetic construct
  source 1..21: mol_type = other DNA
ccggttctgaaggtgttcttg

SEQ ID NO: 148 - DNA, 22 bp, synthetic construct
  source 1..22: mol_type = other DNA
tccggttctgaaggtgttcttg

SEQ ID NO: 149 - DNA, 23 bp, synthetic construct
  source 1..23: mol_type = other DNA
ctccggttctgaaggtgttcttg

SEQ ID NO: 150 - DNA, 24 bp, synthetic construct
  source 1..24: mol_type = other DNA
cctccggttctgaaggtgttcttg

SEQ ID NO: 151 - DNA, 25 bp, synthetic construct
  source 1..25: mol_type = other DNA
gcctccggttctgaaggtgttcttg

SEQ ID NO: 152 - DNA, 26 bp, synthetic construct
  source 1..26: mol_type = other DNA
tgcctccggttctgaaggtgttcttg

SEQ ID NO: 153 - DNA, 20 bp, synthetic construct
  source 1..20: mol_type = other DNA
ccggttctgaaggtgttctt

SEQ ID NO: 154 - DNA, 21 bp, synthetic construct
  source 1..21: mol_type = other DNA
tccggttctgaaggtgttctt

SEQ ID NO: 155 - DNA, 22 bp, synthetic construct
  source 1..22: mol_type = other DNA
ctccggttctgaaggtgttctt

SEQ ID NO: 156 - DNA, 23 bp, synthetic construct
  source 1..23: mol_type = other DNA
cctccggttctgaaggtgttctt

SEQ ID NO: 157 - DNA, 24 bp, synthetic construct
  source 1..24: mol_type = other DNA
gcctccggttctgaaggtgttctt

SEQ ID NO: 158 - DNA, 25 bp, synthetic construct
  source 1..25: mol_type = other DNA
tgcctccggttctgaaggtgttctt

SEQ ID NO: 159 - DNA, 19 bp, synthetic construct
  source 1..19: mol_type = other DNA
ccggttctgaaggtgttct

SEQ ID NO: 160 - DNA, 20 bp, synthetic construct
  source 1..20: mol_type = other DNA
tccggttctgaaggtgttct

SEQ ID NO: 161 - DNA, 21 bp, synthetic construct
  source 1..21: mol_type = other DNA
ctccggttctgaaggtgttct

SEQ ID NO: 162 - DNA, 22 bp, synthetic construct
  source 1..22: mol_type = other DNA
cctccggttctgaaggtgttct

SEQ ID NO: 163 - DNA, 23 bp, synthetic construct
  source 1..23: mol_type = other DNA
gcctccggttctgaaggtgttct

SEQ ID NO: 164 - DNA, 24 bp, synthetic construct
  source 1..24: mol_type = other DNA
tgcctccggttctgaaggtgttct

SEQ ID NO: 165 - DNA, 18 bp, synthetic construct
  source 1..18: mol_type = other DNA
ccggttctgaaggtgttc

SEQ ID NO: 166 - DNA, 19 bp, synthetic construct
  source 1..19: mol_type = other DNA
tccggttctgaaggtgttc

SEQ ID NO: 167 - DNA, 20 bp, synthetic construct
  source 1..20: mol_type = other DNA
ctccggttctgaaggtgttc

SEQ ID NO: 168 - DNA, 21 bp, synthetic construct
  source 1..21: mol_type = other DNA
cctccggttctgaaggtgttc

SEQ ID NO: 169 - DNA, 22 bp, synthetic construct
  source 1..22: mol_type = other DNA
gcctccggttctgaaggtgttc

SEQ ID NO: 170 - DNA, 23 bp, synthetic construct
  source 1..23: mol_type = other DNA
tgcctccggttctgaaggtgttc

SEQ ID NO: 171 - DNA, 25 bp, synthetic construct
  source 1..25: mol_type = other DNA
gttgcctccggttctgaaggtgttc

SEQ ID NO: 172 - RNA, 31 nt, synthetic construct
  source 1..31: mol_type = other RNA
cattcaactgttgcctccggttctgaaggtg

SEQ ID NO: 173 - protein, 12 aa, synthetic construct
  MOD_RES 2: note = misc_feature - Xaa is bAla
  MOD_RES 4: note = misc_feature - Xaa is bAla
  MOD_RES 6: note = misc_feature - Xaa is glucosylated serine
  MOD_RES 8: note = misc_feature - Xaa is bAla
  MOD_RES 10: note = misc_feature - Xaa is bAla
  MOD_RES 12: note = misc_feature - Xaa is bAla
RXRXRXRXRXRX

SEQ ID NO: 174 - protein, 22 aa, synthetic construct
  MOD_RES 2: note = misc_feature - Xaa is 6-aminohexanoic acid
  MOD_RES 5: note = misc_feature - Xaa is bAla
  MOD_RES 8: note = misc_feature - Xaa is 6-aminohexanoic acid
  MOD_RES 16: note = misc_feature - Xaa is 6-aminohexanoic acid
  MOD_RES 18: note = misc_feature - Xaa is bAla
  MOD_RES 20: note = misc_feature - Xaa is 6-aminohexanoic acid
  MOD_RES 22: note = misc_feature - Xaa is bAla
RXRRXRRXRYQFLIRXRXRXRX

SEQ ID NO: 175 - protein, 18 aa, synthetic construct
  MOD_RES 2: note = misc_feature - Xaa is 6-aminohexanoic acid
  MOD_RES 5: note = misc_feature - Xaa is bAla
  MOD_RES 14: note = misc_feature - Xaa is bAla
  MOD_RES 16: note = misc_feature - Xaa is 6-aminohexanoic acid
  MOD_RES 18: note = misc_feature - Xaa is bAla
RXRRXRRFQILYRXRXRX

SEQ ID NO: 176 - protein, 7 aa, synthetic construct
RRRRRRG

SEQ ID NO: 177 - DNA, 21 bp, synthetic construct
  source 1..21: mol_type = other DNA
gctgcccaataccaggtcaac

SEQ ID NO: 178 - DNA, 22 bp, synthetic construct
  source 1..22: mol_type = other DNA
tggtgggagaaatgctgtatgc

SEQ ID NO: 179 - DNA, 20 bp, synthetic construct
  source 1..20: mol_type = other DNA
ttagaggaggtgatggagca

SEQ ID NO: 180 - DNA, 20 bp, synthetic construct
  source 1..20: mol_type = other DNA
gatactaaggactccatcgc

SEQ ID NO: 181 - protein, 16 aa, synthetic construct
  MOD_RES 3: note = misc_feature - Xaa is bAla
  MOD_RES 6: note = misc_feature - Xaa is bAla
  MOD_RES 13: note = misc_feature - Xaa is bAla
  MOD_RES 15: note = misc_feature - Xaa is bAla
ERXRRXRFQILYXRXR

SEQ ID NO: 182 - protein, 18 aa, synthetic construct
  MOD_RES 2: note = misc_feature - Xaa is bAla
  MOD_RES 5: note = misc_feature - Xaa is bAla
  MOD_RES 14: note = misc_feature - Xaa is bAla
  MOD_RES 16: note = misc_feature - Xaa is bAla
  MOD_RES 18: note = misc_feature - Xaa is aminobutyric acid
RXRRXRRFQILYRXHXHX

SEQ ID NO: 183 - protein, 18 aa, synthetic construct
  MOD_RES 2: note = misc_feature - Xaa is bAla
  MOD_RES 5: note = misc_feature - Xaa is bAla
  MOD_RES 14: note = misc_feature - Xaa is bAla
  MOD_RES 16: note = misc_feature - Xaa is bAla
RXRRXRRFQILYRXHXHE

SEQ ID NO: 184 - protein, 18 aa, synthetic construct
  MOD_RES 3: note = misc_feature - Xaa is bAla
  MOD_RES 6: note = misc_feature - Xaa is bAla
  MOD_RES 15: note = misc_feature - Xaa is bAla
  MOD_RES 17: note = misc_feature - Xaa is bAla
ERXRRXRRFQILYRXHXH

SEQ ID NO: 185 - protein, 17 aa, synthetic construct
  MOD_RES 2: note = misc_feature - Xaa is bAla
  MOD_RES 5: note = misc_feature - Xaa is bAla
  MOD_RES 13: note = misc_feature - Xaa is bAla
  MOD_RES 15: note = misc_feature - Xaa is bAla
RXRRXRFQILYRXHXHE

SEQ ID NO: 186 - DNA, 20 bp, synthetic construct
  source 1..20: mol_type = other DNA
caggccattcctctttcagg

SEQ ID NO: 187 - DNA, 21 bp, synthetic construct
  source 1..21: mol_type = other DNA
gaaactttcctcccagttggt

SEQ ID NO: 188 - DNA, 29 bp, synthetic construct
  modified_base 1: mod_base = OTHER; note = misc_feature - Labelled with FAM
  modified_base 9..10: mod_base = OTHER; note = misc_feature - Residues no. 9 and no. 10 are linked through an internal quencher ZEN
  modified_base 29: mod_base = OTHER; note = misc_feature - Labelled with IABkFQ
  source 1..29: mol_type = other DNA
tcaacttcagccatccatttctgtaaggt

SEQ ID NO: 189 - DNA, 24 bp, synthetic construct
  source 1..24: mol_type = other DNA
ctgaatatgaaataatggaggagg

SEQ ID NO: 190 - DNA, 25 bp, synthetic construct
  source 1..25: mol_type = other DNA
cttcagccatccatttctgtaaggt

SEQ ID NO: 191 - DNA, 19 bp, synthetic construct
  modified_base 1: mod_base = OTHER; note = misc_feature - Labelled with FAM
  modified_base 9..10: mod_base = OTHER; note = misc_feature - Residues no. 9 and no. 10 are linked through an internal quencher ZEN
  modified_base 19: mod_base = OTHER; note = misc_feature - Labelled with IABkFQ
  source 1..19: mol_type = other DNA
atgtgattctgtaatttcc

SEQ ID NO: 192 - DNA, 21 bp, synthetic construct
  source 1..21: mol_type = other DNA
cagcagcagcagcagcagcag

SEQ ID NO: 193 - DNA, 31 bp, synthetic construct
  source 1..31: mol_type = other DNA
gctgcccaatgccatcctggagttcctgtaa

SEQ ID NO: 194 - DNA, 22 bp, synthetic construct
  source 1..22: mol_type = other DNA
caatgccatcctggagttcctg

SEQ ID NO: 195 - DNA, 30 bp, synthetic construct
  source 1..30: mol_type = other DNA
ctccaacatcaaggaagatggcatttctag

SEQ ID NO: 196 - DNA, 30 bp, synthetic construct
  source 1..30: mol_type = other DNA
acatcaaggaagatggcatttctagtttgg

SEQ ID NO: 197 - protein, 16 aa, synthetic construct
  MOD_RES 2: note = misc_feature - Xaa is bAla
  MOD_RES 5: note = misc_feature - Xaa is bAla
  MOD_RES 12: note = misc_feature - Xaa is bAla
  MOD_RES 14: note = misc_feature - Xaa is bAla
RXRRXRFQILYXRXRE

SEQ ID NO: 198 - DNA, 31 bp, synthetic construct
  source 1..31: mol_type = other DNA
cattcaactgttgcctccggttctgaaggtg

SEQ ID NO: 199 - protein, 18 aa, synthetic construct
  MOD_RES 2: note = misc_feature - Xaa is bAla
  MOD_RES 5: note = misc_feature - Xaa is bAla
  MOD_RES 14: note = misc_feature - Xaa is bAla
  MOD_RES 16: note = misc_feature - Xaa is bAla
  MOD_RES 18: note = misc_feature - Xaa is bAla
RXRRXRRFQILYRXRXRX

SEQ ID NO: 200 - protein, 17 aa, synthetic construct
  MOD_RES 2: note = misc_feature - Xaa is bAla
  MOD_RES 5: note = misc_feature - Xaa is bAla
  MOD_RES 14: note = misc_feature - Xaa is bAla
  MOD_RES 17: note = misc_feature - Xaa is bAla
RXRRXRRFQILYRXRRX

SEQ ID NO: 201 - protein, 18 aa, synthetic construct
  MOD_RES 2: note = misc_feature - Xaa is bAla
  MOD_RES 5: note = misc_feature - Xaa is bAla
  MOD_RES 14: note = misc_feature - Xaa is bAla
  MOD_RES 16: note = misc_feature - Xaa is bAla
  MOD_RES 18: note = misc_feature - Xaa is bAla
RXRRXRFQILYRRXRXRX

SEQ ID NO: 202 - protein, 18 aa, synthetic construct
  MOD_RES 2: note = misc_feature - Xaa is bAla
  MOD_RES 4: note = misc_feature - Xaa is bAla
  MOD_RES 12: note = misc_feature - Xaa is bAla
  MOD_RES 15: note = misc_feature - Xaa is bAla
  MOD_RES 18: note = misc_feature - Xaa is bAla
RXRXRFQILYRXRRXRRX

SEQ ID NO: 203 - protein, 18 aa, synthetic construct
  MOD_RES 2: note = misc_feature - Xaa is bAla
  MOD_RES 5: note = misc_feature - Xaa is bAla
  MOD_RES 14: note = misc_feature - Xaa is bAla
  MOD_RES 16: note = misc_feature - Xaa is bAla
  MOD_RES 18: note = misc_feature - Xaa is bAla
RXRRXRRYQFLIRXRXRX

SEQ ID NO: 204 - protein, 18 aa, synthetic construct
  MOD_RES 2: note = misc_feature - Xaa is bAla
  MOD_RES 5: note = misc_feature - Xaa is bAla
  MOD_RES 14: note = misc_feature - Xaa is bAla
  MOD_RES 16: note = misc_feature - Xaa is bAla
  MOD_RES 18: note = misc_feature - Xaa is bAla
RXRRXRRILFQYRXRXRX

SEQ ID NO: 205 - protein, 17 aa, synthetic construct
  MOD_RES 2: note = misc_feature - Xaa is bAla
  MOD_RES 5: note = misc_feature - Xaa is bAla
  MOD_RES 13: note = misc_feature - Xaa is bAla
  MOD_RES 15: note = misc_feature - Xaa is bAla
  MOD_RES 17: note = misc_feature - Xaa is bAla
RXRRXRFQILYRXRXRX

SEQ ID NO: 206 - protein, 17 aa, synthetic construct
  MOD_RES 2: note = misc_feature - Xaa is bAla
  MOD_RES 5: note = misc_feature - Xaa is bAla
  MOD_RES 12: note = misc_feature - Xaa is bAla
  MOD_RES 15: note = misc_feature - Xaa is bAla
  MOD_RES 17: note = misc_feature - Xaa is bAla
RXRRXFQILYRXRRXRX

SEQ ID NO: 207 - protein, 16 aa, synthetic construct
  MOD_RES 2: note = misc_feature - Xaa is bAla
  MOD_RES 5: note = misc_feature - Xaa is bAla
  MOD_RES 12: note = misc_feature - Xaa is bAla
  MOD_RES 14: note = misc_feature - Xaa is bAla
  MOD_RES 16: note = misc_feature - Xaa is bAla
RXRRXRFQILYXRXRX

SEQ ID NO: 208 - protein, 16 aa, synthetic construct
  MOD_RES 2: note = misc_feature - Xaa is bAla
  MOD_RES 5: note = misc_feature - Xaa is bAla
  MOD_RES 12: note = misc_feature - Xaa is bAla
  MOD_RES 14: note = misc_feature - Xaa is bAla
  MOD_RES 16: note = misc_feature - Xaa is bAla
RXRRXFQILYRXRXRX

SEQ ID NO: 209 - protein, 18 aa, synthetic construct
  MOD_RES 2: note = misc_feature - Xaa is bAla
  MOD_RES 5: note = misc_feature - Xaa is bAla
  MOD_RES 14: note = misc_feature - Xaa is bAla
  MOD_RES 16: note = misc_feature - Xaa is bAla
  MOD_RES 18: note = misc_feature - Xaa is bAla
RXRRXRRFQILYRXHXHX

SEQ ID NO: 210 - protein, 18 aa, synthetic construct
  MOD_RES 2: note = misc_feature - Xaa is bAla
  MOD_RES 5: note = misc_feature - Xaa is bAla
  MOD_RES 14: note = misc_feature - Xaa is bAla
  MOD_RES 16: note = misc_feature - Xaa is bAla
  MOD_RES 18: note = misc_feature - Xaa is bAla
RXRRXRRFQILYHXHXRX

SEQ ID NO: 211 - protein, 18 aa, synthetic construct
  MOD_RES 2: note = misc_feature - Xaa is bAla
  MOD_RES 5: note = misc_feature - Xaa is bAla
  MOD_RES 14: note = misc_feature - Xaa is bAla
  MOD_RES 16: note = misc_feature - Xaa is bAla
  MOD_RES 18: note = misc_feature - Xaa is bAla
RXRRXRRFQILYHXRXHX

SEQ ID NO: 212 - protein, 18 aa, synthetic construct
  MOD_RES 2: note = misc_feature - Xaa is bAla
  MOD_RES 5: note = misc_feature - Xaa is bAla
  MOD_RES 14: note = misc_feature - Xaa is bAla
  MOD_RES 16: note = misc_feature - Xaa is bAla
  MOD_RES 18: note = misc_feature - Xaa is bAla
RXRRXRRYQFLIRXHXHX

SEQ ID NO: 213 - protein, 18 aa, synthetic construct
  MOD_RES 2: note = misc_feature - Xaa is bAla
  MOD_RES 5: note = misc_feature - Xaa is bAla
  MOD_RES 14: note = misc_feature - Xaa is bAla
  MOD_RES 16: note = misc_feature - Xaa is bAla
  MOD_RES 18: note = misc_feature - Xaa is bAla
RXRRXRRILFQYRXHXHX

SEQ ID NO: 214 - protein, 18 aa, synthetic construct
  MOD_RES 2: note = misc_feature - Xaa is bAla
  MOD_RES 5: note = misc_feature - Xaa is bAla
  MOD_RES 14: note = misc_feature - Xaa is bAla
  MOD_RES 16: note = misc_feature - Xaa is bAla
  MOD_RES 18: note = misc_feature - Xaa is bAla
RXRHXHRFQILYRXRXRX

SEQ ID NO: 215 - protein, 18 aa, synthetic construct
  MOD_RES 2: note = misc_feature - Xaa is bAla
  MOD_RES 4: note = misc_feature - Xaa is bAla
  MOD_RES 5: note = misc_feature - Xaa is bAla
  MOD_RES 14: note = misc_feature - Xaa is bAla
  MOD_RES 16: note = misc_feature - Xaa is bAla
  MOD_RES 18: note = misc_feature - Xaa is bAla
RXRXXHRFQILYRXHXHX

SEQ ID NO: 216 - protein, 17 aa, synthetic construct
  MOD_RES 2: note = misc_feature - Xaa is bAla
  MOD_RES 5: note = misc_feature - Xaa is bAla
  MOD_RES 13: note = misc_feature - Xaa is bAla
  MOD_RES 15: note = misc_feature - Xaa is bAla
  MOD_RES 17: note = misc_feature - Xaa is bAla
RXRRXRFQILYRXHXHX

SEQ ID NO: 217 - protein, 17 aa, synthetic construct
  MOD_RES 2: note = misc_feature - Xaa is bAla
  MOD_RES 5: note = misc_feature - Xaa is bAla
  MOD_RES 13: note = misc_feature - Xaa is bAla
  MOD_RES 15: note = misc_feature - Xaa is bAla
  MOD_RES 17: note = misc_feature - Xaa is bAla
RXRRXRFQILYHXHXHX

SEQ ID NO: 218 - protein, 17 aa, synthetic construct
  MOD_RES 2: note = misc_feature - Xaa is bAla
  MOD_RES 5: note = misc_feature - Xaa is bAla
  MOD_RES 13: note = misc_feature - Xaa is bAla
  MOD_RES 15: note = misc_feature - Xaa is bAla
  MOD_RES 17: note = misc_feature - Xaa is bAla
RXRRXHFQILYRXHXHX

SEQ ID NO: 219 - protein, 17 aa, synthetic construct
  MOD_RES 2: note = misc_feature - Xaa is bAla
  MOD_RES 5: note = misc_feature - Xaa is bAla
  MOD_RES 13: note = misc_feature - Xaa is bAla
  MOD_RES 15: note = misc_feature - Xaa is bAla
  MOD_RES 17: note = misc_feature - Xaa is bAla
HXRRXRFQILYRXHXHX

SEQ ID NO: 220 - protein, 16 aa, synthetic construct
  MOD_RES 2: note = misc_feature - Xaa is bAla
  MOD_RES 5: note = misc_feature - Xaa is bAla
  MOD_RES 12: note = misc_feature - Xaa is bAla
  MOD_RES 14: note = misc_feature - Xaa is bAla
  MOD_RES 16: note = misc_feature - Xaa is bAla
RXRRXFQILYRXHXHX

SEQ ID NO: 221 - protein, 16 aa, synthetic construct
  MOD_RES 2: note = misc_feature - Xaa is bAla
  MOD_RES 5: note = misc_feature - Xaa is bAla
  MOD_RES 12: note = misc_feature - Xaa is bAla
  MOD_RES 14: note = misc_feature - Xaa is bAla
  MOD_RES 16: note = misc_feature - Xaa is bAla
RXRRXRFQILYXHXHX

SEQ ID NO: 222 - protein, 17 aa, synthetic construct
  MOD_RES 2: note = misc_feature - Xaa is bAla
  MOD_RES 5: note = misc_feature - Xaa is bAla
  MOD_RES 13: note = misc_feature - Xaa is bAla
  MOD_RES 15: note = misc_feature - Xaa is bAla
  MOD_RES 17: note = misc_feature - Xaa is bAla
RXRRXRYQFLIHXHXHX

SEQ ID NO: 223 - protein, 17 aa, synthetic construct
  MOD_RES 2: note = misc_feature - Xaa is bAla
  MOD_RES 5: note = misc_feature - Xaa is bAla
  MOD_RES 13: note = misc_feature - Xaa is bAla
  MOD_RES 15: note = misc_feature - Xaa is bAla
  MOD_RES 17: note = misc_feature - Xaa is bAla
RXRRXRILFQYHXHXHX

SEQ ID NO: 224 - protein, 18 aa, synthetic construct
  MOD_RES 2: note = misc_feature - Xaa is bAla
  MOD_RES 5: note = misc_feature - Xaa is bAla
  MOD_RES 14: note = misc_feature - Xaa is bAla
  MOD_RES 16: note = misc_feature - Xaa is bAla
  MOD_RES 18: note = misc_feature - Xaa is bAla
RXRRXRRFQILYHXHXHX

SEQ ID NO: 225 - protein, 14 aa, synthetic construct
  MOD_RES 2: note = misc_feature - Xaa is bAla
  MOD_RES 5: note = misc_feature - Xaa is bAla
  MOD_RES 10: note = misc_feature - Xaa is bAla
  MOD_RES 12: note = misc_feature - Xaa is bAla
  MOD_RES 14: note = misc_feature - Xaa is bAla
RXRRXRWWWXRXRX

SEQ ID NO: 226 - protein, 16 aa, synthetic construct
  MOD_RES 2: note = misc_feature - Xaa is bAla
  MOD_RES 5: note = misc_feature - Xaa is bAla
  MOD_RES 12: note = misc_feature - Xaa is bAla
  MOD_RES 14: note = misc_feature - Xaa is bAla
  MOD_RES 16: note = misc_feature - Xaa is bAla
RXRRXRWWPWWXRXRX

SEQ ID NO: 227 - DNA, 20 bp, synthetic construct
  source 1..20: mol_type = other DNA
tgctcctgtggctgtctcct

SEQ ID NO: 228 - DNA, 21 bp, synthetic construct
  source 1..21: mol_type = other DNA
agcttggctctggcctgtcct

SEQ ID NO: 229 - DNA, 20 bp, synthetic construct
  source 1..20: mol_type = other DNA
accagccactcagccagtga

SEQ ID NO: 230 - DNA, 23 bp, synthetic construct
  source 1..23: mol_type = other DNA
gattgttctagcctcttgattgc